European Patent Application EP 4 372 007 A1, published May 22, 2024. Title: HIF-1a inhibitor. Applicant: NOVELTY NOBILITY INC. The sequence listing filed with the application follows.

SEQUENCE LISTING (30 sequences)

SEQ ID NO: 1 - protein, 11 aa, synthetic construct
  REGION 1..11: note = CDR1 of 2G4 light chain
QSLLHSNGYNY

SEQ ID NO: 2 - skipped

SEQ ID NO: 3 - protein, 8 aa, synthetic construct
  REGION 1..8: note = CDR3 of 2G4 light chain
MQALQTIT

SEQ ID NO: 4 - protein, 8 aa, synthetic construct
  REGION 1..8: note = CDR1 of 2G4 heavy chain
GFTFSRYG

SEQ ID NO: 5 - protein, 8 aa, synthetic construct
  REGION 1..8: note = CDR2 of 2G4 heavy chain
IWYDGTNK

SEQ ID NO: 6 - protein, 11 aa, synthetic construct
  REGION 1..11: note = CDR3 of 2G4 heavy chain
AREDWAEAFDM

SEQ ID NO: 7 - protein, 111 aa, synthetic construct
  REGION 1..111: note = variable domain of 2G4 light chain
DIVMTQSPLSLPVTPGEPASISCRSSQSLLHSNGYNYLDWYLQKPGQSPQLLIYLGSNRASGVPDRFSGSGSGTDFTLKISRVEAEDVGVYYCMQALQTITFGQGTRLEIK

SEQ ID NO: 8 - protein, 118 aa, synthetic construct
  REGION 1..118: note = variable domain of 2G4 heavy chain
QVQLVESGGGVVQPGRSLRLSCAASGFTFSRYGMHWVRQAPGKGLEWVAVIWYDGTNKDYTDSVRGRFTISRDNSKNTLYLQMNSLRAEDTAVYYCAREDWAEAFDMWGQGTTVTVSS

SEQ ID NO: 9 - DNA, 33 bp, synthetic construct
  misc_feature 1..33: note = CDR1 of 2G4 light chain
  source 1..33: mol_type = other DNA
cagagcctcctgcatagtaatggatacaactat

SEQ ID NO: 10 - skipped

SEQ ID NO: 11 - DNA, 24 bp, synthetic construct
  misc_feature 1..24: note = CDR3 of 2G4 light chain
  source 1..24: mol_type = other DNA
atgcaagctctacaaactatcacc

SEQ ID NO: 12 - DNA, 24 bp, synthetic construct
  misc_feature 1..24: note = CDR1 of 2G4 heavy chain
  source 1..24: mol_type = other DNA
ggattcaccttcagtcgctatggc

SEQ ID NO: 13 - DNA, 24 bp, synthetic construct
  misc_feature 1..24: note = CDR2 of 2G4 heavy chain
  source 1..24: mol_type = other DNA
atatggtatgatggaactaataaa

SEQ ID NO: 14 - DNA, 33 bp, synthetic construct
  misc_feature 1..33: note = CDR3 of 2G4 heavy chain
  source 1..33: mol_type = other DNA
gcgagagaagattgggctgaggcttttgatatg

SEQ ID NO: 15 - DNA, 333 bp, synthetic construct
  misc_feature 1..333: note = variable domain of 2G4 light chain
  source 1..333: mol_type = other DNA
gatattgtgatgactcagtctccactctccctgcccgtcacccctggagagccggcctccatctcctgcaggtctagtcagagcctcctgcatagtaatggatacaactatttggattggtacctgcagaagccagggcagtctccacagctcctgatctatttgggttctaatcgggcctccggggtccctgacaggttcagtggcagtggatcaggcacagattttacactgaaaatcagcagagtggaggctgaggatgttggggtttattactgcatgcaagctctacaaactatcaccttcggccaagggacacgactggagattaaa

SEQ ID NO: 16 - DNA, 354 bp, synthetic construct
  misc_feature 1..354: note = variable domain of 2G4 heavy chain
  source 1..354: mol_type = other DNA
caggtgcagctggtggagtctgggggaggcgtggtccagcctgggaggtccctgagactctcctgtgcagcgtctggattcaccttcagtcgctatggcatgcactgggtccgccaggctccaggcaaggggctggagtgggtggcagttatatggtatgatggaactaataaagactatacagactccgtgaggggccgattcaccatctccagagacaattccaagaacacgctgtatcttcaaatgaacagcctgagagccgaggacacggctgtgtattactgtgcgagagaagattgggctgaggcttttgatatgtggggccaagggacaacggtcaccgtctcttca

SEQ ID NO: 17 - DNA, 33 bp, synthetic construct
  misc_feature 1..33: note = CDR1 of 2G4 light chain_optimized codon for CHO
  source 1..33: mol_type = other DNA
cagtccctgctgcactccaacggctacaactac

SEQ ID NO: 18 - skipped

SEQ ID NO: 19 - DNA, 24 bp, synthetic construct
  misc_feature 1..24: note = CDR3 of 2G4 light chain_optimized codon for CHO
  source 1..24: mol_type = other DNA
atgcaggccctgcagaccatcacc

SEQ ID NO: 20 - DNA, 24 bp, synthetic construct
  misc_feature 1..24: note = CDR1 of 2G4 heavy chain_optimized codon for CHO
  source 1..24: mol_type = other DNA
ggcttcaccttctccagatacgga

SEQ ID NO: 21 - DNA, 24 bp, synthetic construct
  misc_feature 1..24: note = CDR2 of 2G4 heavy chain_optimized codon for CHO
  source 1..24: mol_type = other DNA
atttggtacgacggcaccaacaag

SEQ ID NO: 22 - DNA, 33 bp, synthetic construct
  misc_feature 1..33: note = CDR3 of 2G4 heavy chain_optimized codon for CHO
  source 1..33: mol_type = other DNA
gccagagaggattgggccgaagccttcgatatg

SEQ ID NO: 23 - DNA, 333 bp, synthetic construct
  misc_feature 1..333: note = variable domain of 2G4 light chain_optimized codon for CHO
  source 1..333: mol_type = other DNA
gacatcgtgatgacccagtctccactgagcctgcctgtgacacctggcgagcctgcttccatctcctgcagatcctctcagtccctgctgcactccaacggctacaactacctggactggtatctgcagaagcccggccagtctcctcagctgctgatctacctgggctccaacagagcttctggcgtgcccgatagattctccggctctggctctggcaccgacttcaccctgaagatctccagagtggaagccgaggacgtgggcgtgtactactgtatgcaggccctgcagaccatcaccttcggccagggaaccagactggaaatcaag

SEQ ID NO: 24 - DNA, 354 bp, synthetic construct
  misc_feature 1..354: note = variable domain of 2G4 heavy chain_optimized codon for CHO
  source 1..354: mol_type = other DNA
caggtgcagctggtggaatctggtggcggagttgtgcagcctggcagatccctgagactgtcttgtgccgcctccggcttcaccttctccagatacggaatgcactgggtccgacaggcccctggcaaaggattggaatgggtcgccgtgatttggtacgacggcaccaacaaggactacaccgactctgtgcggggcagattcaccatctctcgggacaactccaagaacaccctgtacctgcagatgaactccctgagagccgaggacaccgccgtgtactactgtgccagagaggattgggccgaagccttcgatatgtggggccagggcacaaccgtgaccgtgtcctct

SEQ ID NO: 25 - protein, 238 aa, synthetic construct
  REGION 1..238: note = 2G4 light chain
METDTLLLWVLLLWVPGSTGDIVMTQSPLSLPVTPGEPASISCRSSQSLLHSNGYNYLDWYLQKPGQSPQLLIYLGSNRASGVPDRFSGSGSGTDFTLKISRVEAEDVGVYYCMQALQTITFGQGTRLEIKRTVAAPSVFIFPPSDEQLKSGTASVVCLLNNFYPREAKVQWKVDNALQSGNSQESVTEQDSKDSTYSLSSTLTLSKADYEKHKVYACEVTHQGLSSPVTKSFNRGEC

SEQ ID NO: 26 - protein, 468 aa, synthetic construct
  REGION 1..468: note = 2G4 heavy chain
METDTLLLWVLLLWVPGSTGQVQLVESGGGVVQPGRSLRLSCAASGFTFSRYGMHWVRQAPGKGLEWVAVIWYDGTNKDYTDSVRGRFTISRDNSKNTLYLQMNSLRAEDTAVYYCAREDWAEAFDMWGQGTTVTVSSASTKGPSVFPLAPSSKSTSGGTAALGCLVKDYFPEPVTVSWNSGALTSGVHTFPAVLQSSGLYSLSSVVTVPSSSLGTQTYICNVNHKPSNTKVDKKVEPKSCDKTHTCPPCPAPELLGGPSVFLFPPKPKDTLMISRTPEVTCVVVDVSHEDPEVKFNWYVDGVEVHNAKTKPREEQYNSTYRVVSVLTVLHQDWLNGKEYKCKVSNKALPAPIEKTISKAKGQPREPQVYTLPPSRDELTKNQVSLTCLVKGFYPSDIAVEWESNGQPENNYKTTPPVLDSDGSFFLYSKLTVDKSRWQQGNVFSCSVMHEALHNHYTQKSLSLSPGK

SEQ ID NO: 27 - DNA, 717 bp, synthetic construct
  misc_feature 1..717: note = 2G4 light chain
  source 1..717: mol_type = other DNA
atggaaacagacacactcctcctctgggtcctcctcctctgggtcccaggcagcacaggagatattgtgatgactcagtctccactctccctgcccgtcacccctggagagccggcctccatctcctgcaggtctagtcagagcctcctgcatagtaatggatacaactatttggattggtacctgcagaagccagggcagtctccacagctcctgatctatttgggttctaatcgggcctccggggtccctgacaggttcagtggcagtggatcaggcacagattttacactgaaaatcagcagagtggaggctgaggatgttggggtttattactgcatgcaagctctacaaactatcaccttcggccaagggacacgactggagattaaacgtacggtggctgcaccatctgtcttcatcttcccgccatctgatgagcagttgaaatctggaactgcctctgttgtgtgcctgctgaataacttctatcccagagaggccaaagtacagtggaaggtggataacgccctccaatcgggtaactcccaggagagtgtcacagagcaggacagcaaggacagcacctacagcctcagcagcaccctgacgctgagcaaagcagactacgagaaacacaaagtctacgcctgcgaagtcacccatcagggcctgagctcgcccgtcacaaagagcttcaacaggggagagtgttga

SEQ ID NO: 28 - DNA, 1407 bp, synthetic construct
  misc_feature 1..1407: note = 2G4 heavy chain
  source 1..1407: mol_type = other DNA
atggaaacagacacactcctcctctgggtcctcctcctctgggtcccaggcagcacaggacaggtgcagctggtggagtctgggggaggcgtggtccagcctgggaggtccctgagactctcctgtgcagcgtctggattcaccttcagtcgctatggcatgcactgggtccgccaggctccaggcaaggggctggagtgggtggcagttatatggtatgatggaactaataaagactatacagactccgtgaggggccgattcaccatctccagagacaattccaagaacacgctgtatcttcaaatgaacagcctgagagccgaggacacggctgtgtattactgtgcgagagaagattgggctgaggcttttgatatgtggggccaagggacaacggtcaccgtctcttcagcctccaccaagggcccatcggtcttccccctggcaccctcctccaagagcacctctgggggcacagcggccctgggctgcctggtcaaggactacttccccgaaccggtgacggtgtcgtggaactcaggcgccctgaccagcggcgtgcacaccttcccggctgtcctacagtcctcaggactctactccctcagcagcgtggtgaccgtgccctccagcagcttgggcacccagacctacatctgcaacgtgaatcacaagcccagcaacaccaaggtggacaagaaagttgagcccaaatcttgtgacaaaactcacacatgcccaccgtgcccagcacctgaactcctggggggaccgtcagtcttcctcttccccccaaaacccaaggacaccctcatgatctcccggacccctgaggtcacatgcgtggtggtggacgtgagccacgaagaccctgaggtcaagttcaactggtacgtggacggcgtggaggtgcataatgccaagacaaagccgcgggaggagcagtacaacagcacgtaccgtgtggtcagcgtcctcaccgtcctgcaccaggactggctgaatggcaaggagtacaagtgcaaggtcagcaacaaagccctcccagcccccatcgagaaaaccatctccaaagccaaagggcagccccgagaaccacaggtgtacaccctgcccccatcccgggatgagctgaccaagaaccaggtcagcctgacctgcctggtcaaaggcttctatcccagcgacatcgccgtggagtgggagagcaatgggcagccggagaacaactacaagaccacgcctcccgtgctggactccgacggctccttcttcctctacagcaagctcaccgtggacaagagcaggtggcagcaggggaacgtcttctcatgctccgtgatgcatgaggctctgcacaaccactacacgcagaagagcctctccctgtctccgggtaaatga

SEQ ID NO: 29 - DNA, 717 bp, synthetic construct
  misc_feature 1..717: note = 2G4 light chain_optimized codon for CHO
  source 1..717: mol_type = other DNA
atggaaaccgacacactgctgctgtgggtgctgctcttgtgggtgccaggatctaccggcgacatcgtgatgacccagtctccactgagcctgcctgtgacacctggcgagcctgcttccatctcctgcagatcctctcagtccctgctgcactccaacggctacaactacctggactggtatctgcagaagcccggccagtctcctcagctgctgatctacctgggctccaacagagcttctggcgtgcccgatagattctccggctctggctctggcaccgacttcaccctgaagatctccagagtggaagccgaggacgtgggcgtgtactactgtatgcaggccctgcagaccatcaccttcggccagggaaccagactggaaatcaagcggacagtggccgctccttccgtgttcatcttcccaccttccgacgagcagctgaagtccggcacagcttctgtcgtgtgcctgctgaacaacttctaccctcgggaagccaaggtgcagtggaaggtggacaatgccctgcagtccggcaactcccaagagtctgtgaccgagcaggactccaaggacagcacctacagcctgtcctccacactgaccctgtccaaggccgactacgagaagcacaaggtgtacgcctgcgaagtgacccatcagggcctgtctagccctgtgaccaagtctttcaaccggggcgagtgctga

SEQ ID NO: 30 - DNA, 1407 bp, synthetic construct
  misc_feature 1..1407: note = 2G4 heavy chain_optimized codon for CHO
  source 1..1407: mol_type = other DNA
atggaaaccgacacactgctgctgtgggtgctgctcttgtgggtgccaggatctacaggacaggtgcagctggtggaatctggtggcggagttgtgcagcctggcagatccctgagactgtcttgtgccgcctccggcttcaccttctccagatacggaatgcactgggtccgacaggcccctggcaaaggattggaatgggtcgccgtgatttggtacgacggcaccaacaaggactacaccgactctgtgcggggcagattcaccatctctcgggacaactccaagaacaccctgtacctgcagatgaactccctgagagccgaggacaccgccgtgtactactgtgccagagaggattgggccgaagccttcgatatgtggggccagggcacaaccgtgaccgtgtcctctgcttctaccaagggacccagcgtgttccctctggctccttccagcaagtctacctctggcggaacagctgctctgggctgcctggtcaaggattacttccctgagcctgtgacagtgtcctggaactctggcgctctgacatccggcgtgcacacctttccagctgtgctgcaatcctccggcctgtactctctgtcctccgtcgtgacagtgccttccagctctctgggaacccagacctacatctgcaatgtgaaccacaagccttccaacaccaaggtggacaagaaggtggaacccaagtcctgcgacaagacccacacctgtccaccatgtcctgctccagaactgctcggcggaccttccgtgttcctgtttcctccaaagcctaaggacaccctgatgatctctcggacccctgaagtgacctgcgtggtggtggatgtgtctcacgaggatcccgaagtgaagttcaattggtacgtggacggcgtggaagtgcacaacgccaagaccaagcctagagaggaacagtacaactccacctacagagtggtgtccgtgctgaccgtgctgcaccaggattggctgaacggcaaagagtacaagtgcaaggtgtccaacaaggccctgcctgctcctatcgaaaagaccatctccaaggccaagggccagcctagggaaccccaggtttacaccttgcctccatctcgggacgagctgaccaagaaccaggtgtccctgacctgtctcgtgaagggcttctacccctccgatatcgccgtggaatgggagtctaatggccagcctgagaacaactacaagacaacccctcctgtgctggactccgacggctcattcttcctgtactccaagctgacagtggacaagtccagatggcagcagggcaacgtgttctcctgctccgtgatgcacgaggccctgcacaatcactacacccagaagtccctgtctctgagccccggcaaatga